European Patent Application EP 4 268 583 A1, published November 1, 2023. Title: Method for producing transformed cell or plant of Zea Mays, nucleic acid construct and method for introducing nucleic acid into cell or plant of Zea Mays. Applicant: KANEKA CORPORATION. The sequence listing filed with the application follows.

SEQUENCE LISTING (25 sequences)

SEQ ID NO: 1 - DNA, 693 bp, Zea mays
  CDS (1)..(693)
atggaggcgctgagcgggcgggtaggcgtcaagtgcgggcggtggaaccctacggcggagcaggtgaaggtcctgacggagctcttccgcgcggggctgcggacgcccagcacggagcagatccagcgcatctccacccacctcagcgccttcggcaaggtggagagcaagaacgtcttctactggttccagaaccacaaggcccgcgagcgccaccaccacaagaagcgacgccgcggcgcgtcgtcgtcctcccccgacagcggcagcggcaggggaagcaacaacgaggaagacggccgtggtgccgcctcgcagtcgcacgacgccgacgccgacgccgacctcgtgctgcaaccgccagagagcaagcgggaggccagaagctatggccaccatcaccggctcgtgacatgtaagctgcagcacgcacgtacacatcgctacgtcagggacgtggtggagcagcaggaggcgtcgccgtcgtgggagcggccgacgagggaggtggagacgctagagctcttccccctcaagtcgtacggcgacctcgaggcggcggagaaggtccggtcgtacgtcagaggaagcggcgccaccagcgagcagtgcagggagttgtccttcttcgacgtcgtctccgccggccgggatccgccgctcgagctcaggctctgcagcttcggtccctag

SEQ ID NO: 2 - protein, 230 aa, Zea mays
MEALSGRVGVKCGRWNPTAEQVKVLTELFRAGLRTPSTEQIQRISTHLSAFGKVESKNVFYWFQNHKARERHHHKKRRRGASSSSPDSGSGRGSNNEEDGRGAASQSHDADADADLVLQPPESKREARSYGHHHRLVTCKLQHARTHRYVRDVVEQQEASPSWERPTREVETLELFPLKSYGDLEAAEKVRSYVRGSGATSEQCRELSFFDVVSAGRDPPLELRLCSFGP

SEQ ID NO: 3 - DNA, 1479 bp, Artificial Sequence
  ZmWOX5bX1-GSG2A-sGFPS65T
atggaggcgctgagcgggcgggtaggcgtcaagtgcgggcggtggaaccctacggcggagcaggtgaaggtcctgacggagctcttccgcgcggggctgcggacgcccagcacggagcagatccagcgcatctccacccacctcagcgccttcggcaaggtggagagcaagaacgtcttctactggttccagaaccacaaggcccgcgagcgccaccaccacaagaagcgacgccgcggcgcgtcgtcgtcctcccccgacagcggcagcggcaggggaagcaacaacgaggaagacggccgtggtgccgcctcgcagtcgcacgacgccgacgccgacgccgacctcgtgctgcaaccgccagagagcaagcgggaggccagaagctatggccaccatcaccggctcgtgacatgtaagctgcagcacgcacgtacacatcgctacgtcagggacgtggtggagcagcaggaggcgtcgccgtcgtgggagcggccgacgagggaggtggagacgctagagctcttccccctcaagtcgtacggcgacctcgaggcggcggagaaggtccggtcgtacgtcagaggaagcggcgccaccagcgagcagtgcagggagttgtccttcttcgacgtcgtctccgccggccgggatccgccgctcgagctcaggctctgcagcttcggtcccggaagcggacaacttctcaactttgacttgctaaagttagctggtgatgttgaatctaatcctggaccaatggtgagcaagggcgaggagctgttcaccggggtggtgcccatcctggtcgagctggacggcgacgtaaacggccacaagttcagcgtgtccggcgagggcgagggcgatgccacctacggcaagctgaccctgaagttcatctgcaccaccggcaagctgcccgtgccctggcccaccctcgtgaccaccttcacctacggcgtgcagtgcttcagccgctaccccgaccacatgaagcagcacgacttcttcaagtccgccatgcccgaaggctacgtccaggagcgcaccatcttcttcaaggacgacggcaactacaagacccgcgccgaggtgaagttcgagggcgacaccctggtgaaccgcatcgagctgaagggcatcgacttcaaggaggacggcaacatcctggggcacaagctggagtacaactacaacagccacaacgtctatatcatggccgacaagcagaagaacggcatcaaggtgaacttcaagatccgccacaacatcgaggacggcagcgtgcagctcgccgaccactaccagcagaacacccccatcggcgacggccccgtgctgctgcccgacaaccactacctgagcacccagtccgccctgagcaaagaccccaacgagaagcgcgatcacatggtcctgctggagttcgtgaccgccgccgggatcactcacggcatggacgagctgtacaagtaa

SEQ ID NO: 4 - DNA, 975 bp, Zea mays
atggagacgccacagcagcaatccgccgccgccgccgccgccgccgcccacgggcaggacgacggcgggtcgccgccgatgtcgccggcctccgccgcggcggcggcgctggcgaacgcgcggtggaacccgaccaaggagcaggtggccgtgctggaggggctgtacgagcacggcctgcgcacccccagcgcggagcagatacagcagatcacgggcaggctgcgggagcacggcgccatcgagggcaagaacgtcttctactggttccagaaccacaaggcccgccagcgccagaggcagaagcaggacagcttcgcctacttcagcaggctcctccgccggcccccgccgctgcccgtgctctccatgccccccgcgccaccgtaccatcacgcccgcgtcccggcgccgcccgcgataccgatgccgatggcgccgccgccgcccgctgcatgcaacgacaacggcggcgcgcgtgtgatctacaggaacccattctacgtggctgcgccgcaggcgccccctgcaaatgccgcctactactacccacagccacagcagcagcagcagcagcaggtgacagtcatgtaccagtacccgagaatggaggtagccggccaggacaagatgatgaccagggccgcggcgcaccagcagcagcagcacaacggcgccgggcaacaaccgggacgcgccggccaccccagccgcgagacgctccagctgttcccgctccagcccaccttcgtgctgcggcacgacaaggggcgcgccgccaacggcagtaataacgactccctgacgtcgacgtcgacggcgactgcgacagcgacagcgacagcgacagcgtccgcttccatctccgaggactcggatggcctggagagcggcagctccggcaagggcgtcgaggaggcgcccgcgctgccgttctatgacttcttcgggctccagtcctccggaggccgctga

SEQ ID NO: 5 - DNA, 753 bp, Zea mays
atgaggcttcaccatttccatgtggcttacttggataaagcggcaggctcgccgccgccgtcgtcgtcaccaccatccatctcaccagcatctcacagtcacagctcgtcgtctgctgccaccatcgtccctctggccctccagcaatactgtctacgcccgcttgcgcccaagatctccttccctgaggcgaggaagatggtcgtccttcctgagttcgctcgcgtcaggaatgcttcttcgaggctgctaaactgcacggtgcaagtgccgccgacgacgacgacggtgggtggcacgacgcggtggaacccgtcgccggaccagataagggtgctggagatgctgtaccgcggggggatgcgcacgcccaactcgttccagatcgagcagatcacggaggagctcggcaagtacggccggatcgagggcaagaacgtcttctactggttccagaaccacaaggcccgcgagcgccagaagcagaagcgagctgccctcctcaccctcagcaccaccaccactgcttccacgctgctaccaccagctgctgaaaccaaggagggagtggagacgaaaaaagaagaagcgtgtgaagatgcatcgagccgcaagcggaggtgcagggcctgggaagatgtcgtcgtccatggtggcggcgacgatgccggtacggaggtagctgacgactactacaccgacgacgatgtgaccctggagctcttcccgctgcgtcctgatcaggggaaataa

SEQ ID NO: 6 - DNA, 1200 bp, Zea mays
atgagtgtgcaagtgtggttgtctcctaaacggggtgcctctcttccagtcttcctcaagttatccacttctctctcgatcgaagtcgaagcacaaaccctactgcccgcccacctcccacgtagtgtgtgtgctactcgatcttgtgtccactctcgcccacacacaaacttccacacgaaccaaagattccaatctgaaccaacgttattctgtcgttctccgcctaaccagcaagcagtcgatcgatcgatggagggaagcagaaacagcccggacaggcagtcgtcgggcggcagccctgaggagcgcggaagcggcggtagcggaggccgtggcgccggggagccggtgcggtcgcggtggacgccgaagccggagcagatactgatcctcgagtccatcttcaacagcggcatggtcaacccgcccaaggatgaaaccgtccgcatccgcaagctgctcgagcgcttcggcgccgtcggtgacgccaacgtcttctactggttccagaaccgccgctcccgctcgcgccgccgccagcgccagatgcaggccgccgcggcggcggcggcaacagcggcggcggcctcctctgcggccaacagctctcccggagctagcgcaaccgtcggccttccttctggtgctctacaatatcccttggtcatgagcgggagcgggaccgcctgccagtatgagcagcaggcgagctcctcgtcgtcgtcgggaagcactgggggctcgtctcttgggctgttcgcgctcggagccggggtgcccagcaccggcggtgggttcttccaggagtcgtgtggcgcttcgtcgccactggcgacagggctgatgatgggggacgtggaccgcagtggcggcagcgacgatctcttcgccatctcccggcagatggggttcgcggcggcgagcccagtcgcctcggcttcggtggcgcctccgagcacaacggcacaccaccagcagtattactcatgtcaatcacctacagggacgatcacggtgttcatcaatggagttccaatggaggttcccagtggtccaatagacatgcgagccattttcggccaggacgtgctgctcgtccattccaccggggccctcctcccagtcgacgactatggaattctaacgcagagcttgcagacgggcgaaagctatttcttggtagcaaggccaacttaa

SEQ ID NO: 7 - DNA, 909 bp, Zea mays
atggcggccaatgcgggcggcggtggagcgggaggaggcagcggcagcggcagcgtggctgcgccggcggtgtgccgccccagcggctcgcggtggacgccgacgccggagcagatcaggatgctgaaggagctctactacggctgcggcatccggtcgcccagctcggagcagatccagcgcatcaccgccatgctgcggcagcacggcaagatcgagggcaagaacgtcttctactggttccagaaccacaaggcccgcgagcgccagaagcgccgcctcaccagcctcgacgtcaacgtgcccgccgccggcgcggccgacgccaccaccagccaactcggcgtcctctcgctgtcgtcgccgccgccttcaggcgcggcgcctccctcgcccaccctcggcttctacgccgccggcaatggcggcggatcggctgtgctgctggacacgagttccgactggggcagcagcggcgctgccatggccaccgagacatgcttcctgcaggactacatgggcgtgacggacacgggcagctcgtcgcagtggccacgcttctcgtcgtcggacacgataatggcggcggccgcggcgcgggcggcgacgacgcgggcgcccgagacgctccctctcttcccgacctgcggcgacgacggcggcagcggtagcagcagctacttgccgttctggggtgccgcgtccacaactgccggcgccacttcttccgttgcgatccagcagcaacaccagctgcaggagcagtacagcttttacagcaacagcaacagcacccagctggccggcaccggcaaccaagacgtatcggcaacagcagcagcagccgccgccctggagctgagcctcagctcatggtgctccccttaccctgctgcagggagtatgtga

SEQ ID NO: 8 - DNA, 798 bp, Zea mays
atgccgcagacaccttcgacccgctggtgcccgacgccggagcagctgatgatcctggaggagatgtaccggagcggcgttaggacgcccaacgcggcggagatccagcagatcacggcgcacctggcctactacggccgcatcgagggcaagaacgtcttctactggttccaaaaccacaaggcccgtgagcgccagcggctccgccggcgcctctgcgcccggcaccagcagcagtacgcgcagcagcagcagcaggccaccgcagcagcgccggcttcgagccctaacagcagcgccacccttcttgcacctccggcagcaggcggcagcagcgccccctgtgtgcatccggcggtgatgcagctgcaccatcaccaccacccgtacgcaaccagcttcagcatgccccatctgggctacttggggcagcaggcggcgactgttacgccagtgctcaacccagccgctgccggcatggtggaccttgcaggagcaggagcaggaaatagggctactggtgcaggcggtgcctatggcggtggagctgggttatacaacagctgcagcagcaatcagctggaggtgtgggacgccacagaggcgatggatcactgcaacgccagctgcggtgcggcatcaggcagctctgacgagggtggcgcagctcatctgcagctgccggcatgctgccgccgccctctcaagacattggacctcttccccactaagagcactggactcaaggacgagtgcagcagctccaagtcgtcctcttgctccacatccactaactaa

SEQ ID NO: 9 - DNA, 2728 bp, Zea mays
tggcttcctgatcccctcacttcctcgaatcattctaagaagaaactcaagccgctaccattaggggcagattaattgctgcactttcagataatctaccatggccactgtgaacaactggctcgctttctccctctccccgcaggagctgccgccctcccagacgacggactccacgctcatctcggccgccaccgccgaccatgtctccggcgatgtctgcttcaacatcccccaagattggagcatgaggggatcagagctttcggcgctcgtcgcggagccgaagctggaggacttcctcggcggcatctccttctccgagcagcatcacaagtccaactgcaacttgatacccagcactagcagcacagtttgctacgcgagctcagctgctagcaccggctaccatcaccagctgtaccagcccaccagctccgcgctccacttcgcggactccgtcatggtggcctcctcggccggtgtccacgacggcggttccatgctcagcgcggccgccgctaacggtgtcgctggcgctgccagtgccaacggcggcggcatcgggctgtccatgatcaagaactggctgcggagccaaccggcgcccatgcagccgagggcggcggcggctgagggcgcgcaggggctctctttgtccatgaacatggcggggacgacccaaggcgctgctggcatgccacttctcgctggagagcgcgcacgggcgcccgagagtgtatcgacgtcagcacagggtggtgccgtcgtcgtcacggcgccgaaggaggatagcggtggcagcggtgttgccggtgctctagtagccgtgagcacggacacgggtggcagcggcggcgcgtcggctgacaacacggcaaggaagacggtggacacgttcgggcagcgcacgtcgatttaccgtggcgtgacaaggcatagatggactgggagatatgaggcacatctttgggataacagttgcagaagggaaggacaaactcgtaagggtcgtcaagtctatttaggtggctatgataaagaggagaaagctgctagggcttatgatcttgctgctctgaagtactggggtgccacaacaacaacaaattttccagtgagtaactacgaaaaggagctcgaggacatgaagcacatgacaaggcaggagtttgtagcgtctctgagaaggaagagcagtggtttctccagaggtgcatccatttacaggggagtgactaggcatcaccaacatggaagatggcaagcacggattggacgagttgcagggaacaaggatctttacttgggcaccttcagcacccaggaggaggcagcggaggcgtacgacatcgcggcgatcaagttccgcggcctcaacgccgtcaccaacttcgacatgagccgctacgacgtgaagagcatcctggacagcagcgccctccccatcggcagcgccgccaagcgtctcaaggaggccgaggccgcagcgtccgcgcagcaccaccacgccggcgtggtgagctacgacgtcggccgcatcgcctcgcagctcggcgacggcggagccctagcggcggcgtacggcgcgcactaccacggcgccgcctggccgaccatcgcgttccagccgggcgccgccaccacaggcctgtaccacccgtacgcgcagcagccaatgcgcggcggcgggtggtgcaagcaggagcaggaccacgcggtgatcgcggccgcgcacagcctgcaggacctccaccacttgaacctgggcgcggccggcgcgcacgactttttctcggcagggcagcaggccgccgccgcagctgcgatgcacggcctggctagcatcgacagtgcgtcgctcgagcacagcaccggctccaactccgtcgtctacaacggcggggtcggcgatagcaacggcgccagcgccgttggcagcggcggtggctacatgatgccgatgagcgctgccggagcaaccactacatcggcaatggtgagccacgagcagatgcatgcacgggcctacgacgaagccaagcaggctgctcagatggggtacgagagctacctggtgaacgcggagaacaatggtggcggaaggatgtctgcatgggggaccgtcgtctctgcagccgcggcggcagcagcaagcagcaacgacaacattgccgccgacgtcggccatggcggcgcgcagctcttcagtgtctggaacgacacttaagctacgcgggccggcctggctctccgaatccgaaccgatcgatgcgtcgtaaaacgtacactgacataagtaacaacacttagggttcttcatggagttgttaccagtaagttgttacttgtcatatgttttaagttctcaatttgtagctggaaggaaagctagggtttcttctgaagggtagggtgatggcttgtgaagagtgccacgcatgcacggggttttctccatgatgacggtaccttcacttgctgccattttggggttcaggttcagaagatggataccgagtagcagtattaaccaaaagccatgtttaaatgggatgggtaggaaattgaaccggcaagcttgcttgtaaatggtagctagggtggatgagctgacacgaggtgaaaatgatggcaccttaatggtctagtgtttccattctagagatcaaactgaagcagggagatgcgcaatagttcattcattgcttttgctggttccatttta

SEQ ID NO: 10 - DNA, 1625 bp, Artificial Sequence
  Pnos-ZmWUS-Tpin
acaagccgttttacgtttggaactgacagaaccgcaacgttgaaggagccactcagccgcgggtttctggagtttaatgagctaagcacatacgtcagaaaccattattgcgcgttcaaaagtcgcctaaggtcactatcagctagcaaatatttcttgtcaaaaatgctccactgacgttccataaattcccctcggtatccaattagagtctcatattcactctcaatccaaataatctgcaagatctcgctcaggaaggccgctgagatagaggcatggcggccaatgcgggcggcggtggagcgggaggaggcagcggcagcggcagcgtggctgcgccggcggtgtgccgccccagcggctcgcggtggacgccgacgccggagcagatcaggatgctgaaggagctctactacggctgcggcatccggtcgcccagctcggagcagatccagcgcatcaccgccatgctgcggcagcacggcaagatcgagggcaagaacgtcttctactggttccagaaccacaaggcccgcgagcgccagaagcgccgcctcaccagcctcgacgtcaacgtgcccgccgccggcgcggccgacgccaccaccagccaactcggcgtcctctcgctgtcgtcgccgccgccttcaggcgcggcgcctccctcgcccaccctcggcttctacgccgccggcaatggcggcggatcggctgtgctgctggacacgagttccgactggggcagcagcggcgctgccatggccaccgagacatgcttcctgcaggactacatgggcgtgacggacacgggcagctcgtcgcagtggccacgcttctcgtcgtcggacacgataatggcggcggccgcggcgcgggcggcgacgacgcgggcgcccgagacgctccctctcttcccgacctgcggcgacgacggcggcagcggtagcagcagctacttgccgttctggggtgccgcgtccacaactgccggcgccacttcttccgttgcgatccagcagcaacaccagctgcaggagcagtacagcttttacagcaacagcaacagcacccagctggccggcaccggcaaccaagacgtatcggcaacagcagcagcagccgccgccctggagctgagcctcagctcatggtgctccccttaccctgctgcagggagtatgtgagagcaacgcgagctgccactgctcttcactgatgtctctggaatggaaggaggaggaagtgagcatagcgttggtgcgttgctgtcactgcaggtcgactctagaggatccccgggtaccagacttgtccatcttctggattggccaacttaattaatgtatgaaataaaaggatgcacacatagtgacatgctaatcactataatgtgggcatcaaagttgtgtgttatgtgtaattactagttatctgaataaaagagaaagagatcatccatatttcttatcctaaatgaatgtcacgtgtctttataattctttgatgaaccagatgcatttcattaaccaaatccatatacatataaatattaatcatatataattaatatcaattgggttagcaaaacaaatctagtctaggtgtgttttgcgaatgcggcc

SEQ ID NO: 11 - DNA, 633 bp, Triticum aestivum
atggaggcgctgagcgggcgggtgggagtgaagtgcgggcggtggaacccgacggcggagcaggtgaaggtgctgacggagctgttccgggcggggctgcggacgccgagcaccgagcagatccagcggatctccacccacctcagcgccttcggcaaggtggagagcaagaacgtcttctactggttccagaaccacaaggcccgcgagcgccaccaccacaagaagcgccgccgcgtcgcatcctgctcccccgacagcagcagcaacgatgaagagaccggccgtgccgccgccgccgagcccgccgacctcgtgctccagcctcccgagagcaagcgggaggccggaggctacaaccaccacccccggatcatgacatgctatgtgagggaggtggcggagcaggaagaggcgacgacgtgggagcggccgacgagggaagtggagacgctggagctgttcccgctcaaagcagcctgctacgacctggagctggaggcggacaggttcagccggtatgtgaggagcggcgagcaacagtgcagggagatctccttcttcgacgtggccaccggacgggatccgccgctggagctcaggctctgcagcttcgatcggtatctggtctaa

SEQ ID NO: 12 - DNA, 603 bp, Oryza sativa
atggaggctcttagcgggcgagtgggggtgaagtgtgggcggtggaacccgacggcggagcaggtgaaggtcctgacggagctgttccgagcggggttgcggacgccgagcacggagcagatccagcgcatctccactcacctcagcgcattcggcaaggtggagagcaagaacgtcttctactggttccagaaccacaaggcccgcgagcgccaccaccacaagaagcgccgccgcggcgcctcctcccccgacagcggcagcaacgatgacgatggccgcgccgcagcccacgagggcgacgccgacctcgtcctgcagcctcctgagagcaagcgggaggccagaagctacggccatcatcaccggctcatgacatgctacgtgagggatgtggtggagacggaagcgatgtgggagcggccgacgagggaggtggaaacgctggagctgttcccactcaagtcgtatgacctcgaggtggacaaggtccggtatgtgaggggcggcggtggcgagcagtgcagggagatctcgttcttcgacgtcgctgccggccgggatccgccgctggagctcaggctttgcagcttcggcctctag

SEQ ID NO: 13 - DNA, 708 bp, Zea mays
atggacacggaggcgccgagcgggcgggtgggcgtcaagtgcgggcggtggaacccgacgccggagcaggtgaaggtcctgacggagctcttccgcgcggggctgcggacgcccagcacggaccagatccagcgcatctccgcccacctcggcgccttcggcaaggtggagagcaagaacgtcttctactggttccagaaccacaaggcccgcgagcgccaccaccacaagaagaagaagcgccgccgacgcggcgcggcaatggcatcgtcgtcctcccccgacagcggcagcggcagcgggagcagcgaggaagacggccgtgttgccgccgccgccgacgccgacctcgtgctgcaaccatcgccgggaagaagcaaaagcaaacgggaggccagaagaagctacggcggcggccaccatcgccggctcgttacatgtaagcagctagcgcacacacatcgctacgtcagggacgttgtggagcagcaggaggaggacacgtgggagcggccgacgagggaggcggtggagactctggagctcttccccctcaagtcgtacgtcgacctcgaggcggagaaggtccggcggtacgtcgtcagggccggcgccagcgagcagtgcagggacttctccttcttcgacgtgtccggcggtcgggatccgccgcttcttgagcttaggctctgcagcttcggtccctag

SEQ ID NO: 14 - DNA, 663 bp, Zea mays
  CDS (1)..(663)
atggaggcgctgagcgggcgggtaggcgtcaagtgcgggcggtggaaccctacggcggagcaggtgaaggtcctgacggagctcttccgcgcggggctgcggacgcccagcacggagcagatccagcgcatctccacccacctcagcgccttcggcaaggtggagagcaagaacgtcttctactggttccagaaccacaaggcccgcgagcgccaccaccacaagaagcgccgccgcggcgcgtcgtcgtcctcccccgacagcggcagcggcaggggaagcaacaacgaggaagacggccgtggtgccgcctcgcagtcgcacgacgccgacgccgacgccgacctcgtgctgcaaccgccagagagcaagcgggaggccagaagctatggccaccatcaccggctcgtgacatgctacgtcagggacgtggtggagcagcaggaggcgtcgccgtcgtgggagcggccgacgagggaggtggagacgctagagctcttccccctcaagtcgtacggcgacctcgaggcggcggagaaggtccggtcgtacgtcagaggcatcgccgccaccagcgagcagtgcagggagttgtccttcttcgacgtctccgccggccgggatccgccgctcgagctcaggctctgcagcttcggtccctag

SEQ ID NO: 15 - protein, 220 aa, Zea mays
MEALSGRVGVKCGRWNPTAEQVKVLTELFRAGLRTPSTEQIQRISTHLSAFGKVESKNVFYWFQNHKARERHHHKKRRRGASSSSPDSGSGRGSNNEEDGRGAASQSHDADADADLVLQPPESKREARSYGHHHRLVTCYVRDVVEQQEASPSWERPTREVETLELFPLKSYGDLEAAEKVRSYVRGIAATSEQCRELSFFDVSAGRDPPLELRLCSFGP

SEQ ID NO: 16 - DNA, 1057 bp, Artificial Sequence
  P35SIcat
agattagccttttcaatttcagaaagaatgctaacccacagatggttagagaggcttacgcagcaggtctcatcaagacgatctacccgagcaataatctccaggaaatcaaataccttcccaagaaggttaaagatgcagtcaaaagattcaggactaactgcatcaagaacacagagaaagatatatttctcaagatcagaagtactattccagtatggacgattcaaggcttgcttcacaaaccaaggcaagtaatagagattggagtctctaaaaaggtagttcccactgaatcaaaggccatggagtcaaagattcaaatagaggacctaacagaactcgccgtaaagactggcgaacagttcatacagagtctcttacgactcaatgacaagaagaaaatcttcgtcaacatggtggagcacgacacacttgtctactccaaaaatatcaaagatacagtctcagaagaccaaagggcaattgagacttttcaacaaagggtaatatccggaaacctcctcggattccattgcccagctatctgtcactttattgtgaagatagtggaaaaggaaggtggctcctacaaatgccatcattgcgataaaggaaaggccatcgttgaagatgcctctgccgacagtggtcccaaagatggacccccacccacgaggagcatcgtggaaaaagaagacgttccaaccacgtcttcaaagcaagtggattgatgtgatatctccactgacgtaagggatgacgcacaatcccactatccttcgcaagacccttcctctatataaggaagttcatttcatttggagagaacacgggggactctagaggatccccgatccctacagggtaaatttctagtttttctccttcattttcttggttaggacccttttctctttttatttttttgagctttgatctttctttaaactgatctattttttaattgattggttatggtgtaaatattacatagctttaactgataatctgattactttatttcgtgtgtctatgatgatgatgatagttacag

SEQ ID NO: 17 - DNA, 1077 bp, Artificial Sequence
  PPLTP
ttaccctagctccctgcggctgttacgcggtcccccatcaatcttctgttcttgcggttgtagcctgtgtaacagtgctagagtatgtatgataaataggttttaagtctgcttacatgacattttttattgtggaagagacatataaaaattagagagagtggttctcatgcaacggcggacggcccggtgctaaaagagcttcaagacaaaataatgaaacaggaagagagtagatttatctaagagccaactttattatatgaatgtgtttattgttggctttagatgatatggtaaggagttagagctaataatagataggctctattattattattattaattaaactcgctctaaggaggaaagtgggaggaagggacgaggacgaagactactggaagcatcgtgcatggatgatggatgtggtgtctcttaatgtaggtggccggaggatgtacgtgttaattgcgcgataagcactcagatccaaccgcaaactacctccacactgacacactgatagagagaaagagagacctccgacgactgccgccgcagatgagccacgtacgtatacgacgtctgccggccggctcaggctgccgccatcaccctgctcgaaagtcgcgttaggcggcgccagctacataggagtatctagtctagccagttagtatactactactgcgctgatgatgaattaactctgcatagatactgtacttgcctccctccaacacccaaccacctcctgctcggctcttaataacttggacacggatcgatgccatccaaggaagaacacgacgacgacgacggaacatccaccatgcaagcttgcatccatacgccgatacgcgtgcatccatccatccaccattatttccattttccaccgatcacacgtacacaggcctatttaaggagcgacatcccactgcaactctcctcaccactcatcaccagctagctctagcaaagcacttgccatctaccgaccgccgcattccaaacagcccgacgagctagcagagcggcaggcacctccctcctcaaggaacctgcaggtcgac

SEQ ID NO: 18 - DNA, 60 bp, Artificial sequence
  DNA encoding 2A peptide derived from foot-and-mouth disease virus (FMDV)
  CDS (1)..(60)
caacttctcaactttgacttgctaaagttagctggtgatgttgaatctaatcctggacca

SEQ ID NO: 19 - protein, 20 aa, Artificial sequence
  2A peptide derived from foot-and-mouth disease virus (FMDV)
QLLNFDLLKLAGDVESNPGP

SEQ ID NO: 20 - DNA, 32 bp, Artificial Sequence
  forward primer for amplifying DNA from RB to LB in pLC41
gactagtcgacaagcagatcacgcttttcgac

SEQ ID NO: 21 - DNA, 32 bp, Artificial Sequence
  reverse primer for amplifying DNA from RB to LB in pLC41
gactagtctccaagagacggttacacaaacgg

SEQ ID NO: 22 - DNA, 27 bp, Artificial Sequence
  forward primer for amplifying DNA from gentamycin gene to T-DNA
gatatcccgggttgacataagcctgtt

SEQ ID NO: 23 - DNA, 23 bp, Artificial Sequence
  reverse primer for amplifying DNA from gentamycin gene to T-DNA
ctccaagagacggttacacaaac

SEQ ID NO: 24 - DNA, 24 bp, Artificial Sequence
  forward primer for amplifying spectinomycin-resistant gene
agctctctaacgcttgagttaagc

SEQ ID NO: 25 - DNA, 21 bp, Artificial Sequence
  reverse primer for amplifying spectinomycin-resistant gene
cgtttcggtgatgacggtgaa